European Patent Specification EP 3 431 597 B1, published January 21, 2026. Title: Immune cells expressing immune-regulatory factors, and Vectors. Applicant: YAMAGUCHI UNIVERSITY. The sequence listing filed with the application follows.

SEQUENCE LISTING (14 sequences)

SEQ ID NO: 1 - protein, 177 aa, artificial
  human IL-7
  Inventor: Tamada, Koji Inventor: Sakoda, Yukimi Inventor: Adachi, Keishi
MFHVSFRYIFGLPPLILVLLPVASSDCDIEGKDGKQYESVLMVSIDQLLDSMKEIGSNCLNNEFNFFKRHICDANKEGMFLFRAARKLRQFLKMNSTGDFDLHLLKVSEGTTILLNCTGQVKGRKPAALGEAQPTKSLEENKSLKEQKKLNDLCFLKRLLQEIKTCWNKILMGTKEH

SEQ ID NO: 2 - protein, 98 aa, artificial
  human CCL19
MALLLALSLLVLWTSPAPTLSGTNDAEDCCLSVTQKPIPGYIVRNFHYLLIKDGCRVPAVVFTTLRGRQLCAPPDQPWVERIIQRLQRTSAKMKRRSS

SEQ ID NO: 3 - DNA, 22 bp, artificial
  5'-R primer
gtctaccaggcattcgcttcat

SEQ ID NO: 4 - DNA, 24 bp, artificial
  3-TRa-C primer
tcagctggaccacagccgcagcgt

SEQ ID NO: 5 - DNA, 21 bp, artificial
  3-TRb-C1 primer
tcagaaatcctttctcttgac

SEQ ID NO: 6 - DNA, 24 bp, artificial
  3-TRbeta-C2 primer
ctagcctctggaatcctttctctt

SEQ ID NO: 7 - protein, 8 aa, artificial
  2A peptide cleavage region
  MISC_FEATURE (2)..(2): Val or Ile
  MISC_FEATURE (4)..(4): any amino acid
DXEXNPGP

SEQ ID NO: 8 - protein, 25 aa, artificial
  2Apeptide(F2A)
GSGVKQTLNFDLLKLAGDVESNPGP

SEQ ID NO: 9 - DNA, 1674 bp, artificial
  anti-FITC CAR
atggagttgcctgttaggttgttggtgctgatgttctggattcctgcttccagcagtgatgtcgtgatgacccaaactccactctccctgcctgtcagtcttggagatcaagcctccatctcttgcagatctagtcagagccttgtacacagtaatggaaacacctatttacgttggtacctgcagaagccaggccagtctccaaaggtcctgatctacaaagtttccaaccgattttctggggtcccagacaggttcagtggcagtggatcagggacagatttcacactcaagatcagcagagtggaggctgaggatctgggagtttatttctgctctcaaagtacacatgttccgtggacgttcggtggaggcaccaagctggaaatcaaaagtagtgctgatgatgctaagaaggatgctgctaagaaggatgatgctaagaaggatgatgctaagaaggatggtgaggtgaagctggatgagactggaggaggcttggtgcaacctgggaggcccatgaaactctcctgtgttgcctctggattcacttttagtgactactggatgaactgggtccgccagtctccagagaaaggactggagtgggtagcacaaattagaaacaaaccttataattatgaaacatattattcagattctgtgaaaggcagattcaccatctcaagagatgattccaaaagtagtgtctacctgcaaatgaacaacttaagagttgaagacatgggtatctattactgtacgggttcttactatggtatggactactggggtcaaggaacctcagtcaccgtctccgcggccgcagtcgtgccagtccttcagaaagtgaactctactactaccaagccagtgctgcgaactccctcacctgtgcaccctaccgggacatctcagccccagagaccagaagattgtcggccccgtggctcagtgaaggggaccggattggacttcgcctgtgatatttacatctgggcacccttggccggaatctgcgtggcccctctgctgtccttgatcatcactctcatctgctaccacaggagccgaaatagtagaaggaacagactccttcaaagtgactacatgaacatgactccccggaggcctgggctcactcgaaagccttaccagccctacgcccctgccagagactttgcagcgtaccgccccaaatggatcaggaaaaaattcccccacatattcaagcaaccatttaagaagaccactggagcagctcaagaggaagatgcttgtagctgccgatgtccacaggaagaagaaggaggaggaggaggctatgagctgagagcaaaattcagcaggagtgcagagactgctgccaacctgcaggaccccaaccagctctacaatgagctcaatctagggcgaagagaggaatatgacgtcttggagaagaagcgggctcgggatccagagatgggaggcaaacagcagaggaggaggaacccccaggaaggcgtatacaatgcactgcagaaagacaagatggcagaagcctacagtgagatcggcacaaaaggcgagaggcggagaggcaaggggcacgatggcctttaccagggtctcagcactgccaccaaggacacctatgatgccctgcatatgcagaccctggcccctcgctaa

SEQ ID NO: 10 - DNA, 146 bp, artificial
  F2A-MCS
ggaagcggagtgaaacagactttgaattttgaccttctcaagttggcgggagacgtggagtccaaccctggaccatgcataaaaagcttaaaccagttaactggaaaacgcgtaaagtcgacaaaggccaaaaaggccaacgtacg

SEQ ID NO: 11 - DNA, 864 bp, artificial
  mouseIL-7-F2A-mouseCCL19
atgttccatgtttcttttagatatatctttggaattcctccactgatccttgttctgctgcctgtcacatcatctgagtgccacattaaagacaaagaaggtaaagcatatgagagtgtactgatgatcagcatcgatgaattggacaaaatgacaggaactgatagtaattgcccgaataatgaaccaaacttttttagaaaacatgtatgtgatgatacaaaggaagctgcttttctaaatcgtgctgctcgcaagttgaagcaatttcttaaaatgaatatcagtgaagaattcaatgtccacttactaacagtatcacaaggcacacaaacactggtgaactgcacaagtaaggaagaaaaaaacgtaaaggaacagaaaaagaatgacgcatgtttcctaaagagactactgagagaaataaaaacttgttggaataaaattttgaagggcagtataggaagcggagtgaaacagactttgaattttgaccttctcaagttggcgggagacgtggagtccaaccctggacctatggccccccgtgtgaccccactcctggccttcagcctgctggttctctggaccttcccagccccaactctggggggtgctaatgatgcggaagactgctgcctgtctgtgacccagcgccccatccctgggaacatcgtgaaagccttccgctaccttcttaatgaagatggctgcagggtgcctgctgttgtgttcaccacactaaggggctatcagctctgtgcacctccagaccagccctgggtggatcgcatcatccgaagactgaagaagtcttctgccaagaacaaaggcaacagcaccagaaggagccctgtgtcttga

SEQ ID NO: 12 - DNA, 783 bp, artificial
  anti-humanCD20 scFv
atggactggacctggcggatcctgttcctggtggctgctgctacaggcgcccacagccagatcgtgctgtctcagtctcccgccatcctgtctgctagccctggcgagaaagtgaccatgacctgcagagccagcagcagcgtgtcctacatccactggttccagcagaagcccggcagcagccccaagccttggatctacgccacaagcaacctggcctctggcgtgccagtgcggtttagcggctctggctctggcaccagctacagcctgaccatcagcagagtggaagccgaggacgccgccacctactactgtcagcagtggaccagcaacccccccacattcggcggaggcaccaagctggaaatcaagggcggaggcggatctggcggcggaggatctgggggaggcggctctcaggtgcagctgcagcagcctggcgctgagctcgtgaaacctggcgcctccgtgaagatgagctgcaaggccagcggctacaccttcacaagctacaacatgcactgggtcaagcagacccctggcagaggcctggaatggatcggcgctatctaccccggcaacggcgacacctcctacaaccagaagttcaagggcaaggccaccctgaccgccgacaagagcagcagcacagcctacatgcagctgtcctccctgaccagcgaggacagcgccgtgtactactgcgccagatctacctactacggcggcgactggtacttcaacgtgtggggcgctggcaccaccgtgaccgtgtctgct

SEQ ID NO: 13 - DNA, 1665 bp, artificial
  Mouse Il-7-F2A-mouseCCL19-F2A-eGFP
atggtccacgtctccttcagatacatcttcggcatcccccccctgatcctggtcctcctgcctgtcacctccagcgaatgtcatatcaaggacaaagagggcaaggcttatgagagcgtcctgatgatctccattgatgagctggataagatgaccggcaccgacagcaactgtcccaacaatgagcccaacttctttagaaagcacgtgtgtgacgataccaaggaggctgccttcctgaacagggccgccagaaagctgaagcagttcctgaagatgaacatttccgaggagttcaacgtgcacctcctcaccgtgagccagggcacccagacactggtcaattgcacctccaaggaggagaagaacgtgaaagagcagaaaaagaatgatgcttgtttcctcaagaggctgctgagggagatcaagacctgttggaataagatcctgaaaggcagcatcggcagcggagtcaagcaaaccctgaacttcgacctgctgaaactggccggagatgtggagagcaatcccggccctatggcccccagagtcacccctctgctggccttcagcctgctcgtgctgtggaccttccccgctcccaccctgggcggcgccaatgatgctgaggactgttgcctctccgtgacccagaggcccatccctggaaacatcgtcaaagccttcaggtacctgctcaacgaagacggatgtagggtgcctgccgtggtgttcacaacactgagaggctaccagctctgcgcccctcctgatcagccctgggtcgacagaatcatcagaaggctgaagaagtccagcgccaagaacaaaggcaatagcacaaggagaagccctgtgagcgaattcggaagcggagtgaaacagactttgaattttgaccttctcaagttggcgggagacgtggagtccaaccctggaccatgcatggtgagcaagggcgaggagctgttcaccggggtggtgcccatcctggtcgagctggacggcgacgtaaacggccacaagttcagcgtgtccggcgagggcgagggcgatgccacctacggcaagctgaccctgaagttcatctgcaccaccggcaagctgcccgtgccctggcccaccctcgtgaccaccctgacctacggcgtgcagtgcttcagccgctaccccgaccacatgaagcagcacgacttcttcaagtccgccatgcccgaaggctacgtccaggagcgcaccatcttcttcaaggacgacggcaactacaagacccgcgccgaggtgaagttcgagggcgacaccctggtgaaccgcatcgagctgaagggcatcgacttcaaggaggacggcaacatcctggggcacaagctggagtacaactacaacagccacaacgtctatatcatggccgacaagcagaagaacggcatcaaggtgaacttcaagatccgccacaacatcgaggacggcagcgtgcagctcgccgaccactaccagcagaacacccccatcggcgacggccccgtgctgctgcccgacaaccactacctgagcacccagtccgccctgagcaaagaccccaacgagaagcgcgatcacatggtcctgctggagttcgtgaccgccgccgggatcactctcggcatggacgagctgtacaagtaa

SEQ ID NO: 14 - protein, 554 aa, artificial
  Mouse Il-7-F2A-mouse CCL19-2A-eGFP amino acid
MVHVSFRYIFGIPPLILVLLPVTSSECHIKDKEGKAYESVLMISIDELDKMTGTDSNCPNNEPNFFRKHVCDDTKEAAFLNRAARKLKQFLKMNISEEFNVHLLTVSQGTQTLVNCTSKEEKNVKEQKKNDACFLKRLLREIKTCWNKILKGSIGSGVKQTLNFDLLKLAGDVESNPGPMAPRVTPLLAFSLLVLWTFPAPTLGGANDAEDCCLSVTQRPIPGNIVKAFRYLLNEDGCRVPAVVFTTLRGYQLCAPPDQPWVDRIIRRLKKSSAKNKGNSTRRSPVSEFGSGVKQTLNFDLLKLAGDVESNPGPCMVSKGEELFTGVVPILVELDGDVNGHKFSVSGEGEGDATYGKLTLKFICTTGKLPVPWPTLVTTLTYGVQCFSRYPDHMKQHDFFKSAMPEGYVQERTIFFKDDGNYKTRAEVKFEGDTLVNRIELKGIDFKEDGNILGHKLEYNYNSHNVYIMADKQKNGIKVNFKIRHNIEDGSVQLADHYQQNTPIGDGPVLLPDNHYLSTQSALSKDPNEKRDHMVLLEFVTAAGITLGMDELYK